European Patent Specification EP 4 036 106 B1, published June 10, 2026. Title: MNEP MONOMER VARIANT AND APPLICATION THEREOF. Applicant: QITAN TECHNOLOGY LTD., BEIJING. The sequence listing filed with the application follows.

SEQUENCE LISTING (17 sequences)

SEQ ID NO: 1 - protein, 191 aa, Artificial Sequence
  Mnep monomer variant
MGLDNELSLVDGKDRTLTIQQWDTFLNGVFPLDRNRLTREWFHSGKAKYIVSGPGAEDFEGALELGYQVGFPWSLGVGINFSYTTPNVALSKFPLFGITGIGGKLPVIGEIATPPLFPGASISADLGNGPGIQEVATFSTEVAGPEGAVAVSNAHGTVTGAAGGVLLRPFARLVSSLGDSVTTYGEPWNMN

SEQ ID NO: 2 - DNA, 576 bp, Artificial Sequence
  the nucleotide sequence encoding the Mnep monomer variant
atgggcttagataacgaactgtctttagtggatggcaaagatcgcactttaaccattcagcagtgggacacctttctgaacggtgtgtttccgctggatcgcaaccgtttaacccgcgagtggtttcacagcggcaaagccaaatatattgtgagcggcccgggtgcagaagactttgaaggcgtgctggagctgggctatcaagttggttttccgtggagtctgggcgtgggcatcaactttagctacaccaccccgaatgtggcactgagtaaatttccgctgtttggcattaccggcattggcggcaaactgccggtgattggcgaaattgcaaccccgccgctgtttccgggtgcaagcattagcgccgatttaggtaacggtccgggcattcaagaagttgccacctttagcaccgaagtggctggtccggaaggtgccgttgccgtgagcaatgctcatggcactgtgactggtgccgctggtggcgttttactgcgcccgtttgcccgtttagtgagcagtctgggtgatagcgtgaccacctatggcgaaccgtggaatatgaactaa

SEQ ID NO: 3 - protein, 863 aa, Artificial Sequence
  helicase EF8813-1
MGSSHHHHHHSSGLVPRGSHMKIESLDLPDEVKQFYLDSGILELYPPQAEAVEKGLLEGRNLLAAIPTASGKTLLAELAMLKSILNGGKALYIVPLRALASEKFKRFREFSKLGIRVGISTGDYDLRDEGLGVNDIIVATSEKTDSLLRNETVWMQEISVVVADEVHLIDSPDRGPTLEITLAKLRKMNPSCQILALSATIGNADELAAWLEAGLVLSEWRPTELREGVFFNGTFYCKDREKSIEQSTKDEAVNLVLDTLREDGQCLVFENSRKNCMAFAKKASSAVKKILSAEDKEALAEIADEVLENSETDTSAALAACIRSGTAFHHAGLTTPLRELVEDGFRAGKIKLISSTPTLAAGLNLPARRVVIRSYRRYSSEDGMQPIPVIEYKQMAGRAGRPRLDPYGEAVLVAKSYEEFVFLFRNYIEADAEDIWSKLGTENALRTHVLSTISNGFARTKEELMEFLEATFFAFQYSNFGLSTVVDECLNFLRQEEMLEKTDTLISTSFGKLVSKLYIDPLSAARIVKGLKEAKILTELTLLHLVCSTPDMRLLYMRNQDYQDINDYVIAHADEFVRVPSPFNYTEYEWFLGEVKTSLLLVDWIHEKSENEICLKFGIGEGDIHAIADIAEWLMHVTAQLARLLELKGAKEAAELEKRIHYGASPELMDLLDIRGIGRMRARKLYESGFRSSAELAGADPVKVAALLGPKIADRIFKQIGRREVLPEIAEPTLPEKSPSSGQKTINDYGTGGGGSWKEWLERKVGEGRARRLIEYFGSAGEVGKLVENAEVSKLLEVPGIGDEAVARLVPGYKTLRDAGLTPAEAERVLKRYGSVSKVQEGATPDELRELGLGDAKIARILG

SEQ ID NO: 4 - DNA, 2592 bp, Artificial Sequence
  helicase EF8813-1
atgggcagcagccatcatcatcatcatcacagcagcggcctggtgccgcgcggcagccatatgaagatcgaaagcctggacctgccggacgaagttaaacagttttacctggatagcggtattttagaactgtacccgccgcaggcagaagcagtagaaaaaggcctgttagaaggacgtaatctgctggcagcaattccgaccgcaagcggtaagacactgctggctgaattagcaatgctgaaaagcatactgaatgggggaaaagcactgtatattgttccgctgagagcactggcatcagaaaaatttaaacgttttagagagttcagcaagttaggtataagagtgggtattagcacaggagactatgacctgagagatgaaggtctgggtgttaatgatattattgtggcaacaagcgaaaaaaccgatagcctgctgcgtaatgaaaccgtttggatgcaggaaattagcgttgttgttgcagatgaagttcatctgattgatagcccggatcgtggtccgaccctggaaattaccctggcaaaactgcgtaaaatgaatccgagctgtcagattctggcactgagcgcaaccattggtaatgcagatgaactggcagcatggctggaagcaggtctggttctgagcgaatggcgtccgaccgaactgcgtgaaggtgttttttttaatggtacattttattgtaaagatcgtgaaaaaagcattgaacagagcaccaaagatgaagcagttaatctggttctggataccctgcgtgaagatggtcagtgtctggtttttgaaaatagccgtaaaaattgtatggcatttgcaaaaaaagcaagcagcgcagttaaaaaaattctgagcgcagaagataaagaagcactggcagaaattgcagatgaagttctggaaaatagcgaaaccgataccagcgcagcactggcagcatgtattcgtagcggtacagcatttcatcatgcaggtctgaccaccccgctgcgtgaactggttgaagatggttttcgtgcaggtaaaattaaactgattagcagcaccccgaccctggcagcaggtctgaatctgccggcacgtcgtgttgttattcgtagctatcgtcgttatagcagcgaagatggtatgcagccgattccggttattgaatataaacagatggcaggtcgtgcaggtcgtccgcgtctggacccttatggtgaagcagttctggttgcaaaaagctatgaagaatttgtttttctgtttcgtaattatattgaagcagatgcagaagatatttggagcaaactgggtacagaaaatgcactgcgtacccatgttctgagcaccattagcaatggttttgcacgtaccaaagaagaactgatggaatttctggaagcaaccttttttgcatttcagtatagcaattttggtctgagcaccgttgttgatgaatgtctgaattttctgcgtcaggaagaaatgctggaaaaaaccgataccctgattagcaccagctttggtaaactggttagcaaactgtatattgatccgctgagcgcagcacgtattgttaaaggtctgaaagaagcaaaaattctgaccgaactgaccctgctgcatctggtttgtagcaccccggatatgcgtctgctgtatatgcgtaatcaggattatcaggatattaatgattatgttattgcacatgcagatgaatttgttcgtgttccgagcccgtttaattataccgaatatgaatggtttctgggtgaagttaaaaccagcctgctgctggttgattggattcatgaaaaaagcgaaaatgaaatttgtctgaaatttggtattggtgaaggtgatattcatgcaattgcagatattgcagaatggctgatgcatgttaccgcacagctggcacgtctgctggaactgaaaggtgcaaaagaagcagcagaactggaaaaacgtattcattatggtgcaagcccggaactgatggatctgctggatattcgtggtattggtcgtatgcgtgcacgtaaactgtatgaaagcggttttcgtagcagcgcagaactggcaggtgcagatccggttaaagttgcagcactgctgggtccgaaaattgcagatcgtatttttaaacagattggtcgtcgtgaagttctgccggaaattgcagaaccgaccctgccggaaaaaagcccgagcagcggtcagaaaaccattaatgattatggtaccggtggaggcggttcctggaaggaatggctggagcgtaaggttggcgagggccgtgcgcgtcgcctgatcgagtatttcggcagcgcgggtgaggttggcaaattggtcgagaatgcggaagtcagcaaattgctggaagttccgggtatcggcgacgaggctgtggctcgcctggtgccgggttataagaccctgcgcgatgccggtctgaccccggcagaagcagagcgcgtgctgaagcgctacggcagcgtcagcaaagtgcaggaaggcgcaacgccggacgaattgcgcgagttaggtctgggcgacgccaagattgcccgcattctgggttaa

SEQ ID NO: 5 - DNA, 54 bp, Artificial Sequence
  X2
tggtttttgtttgtttttagaatttttttacactaccactgctagcatttttca

SEQ ID NO: 6 - DNA, 45 bp, Artificial Sequence
  X2
tttctcactatcccgttctcattggtgcaccatctttttttggtt

SEQ ID NO: 7 - DNA, 15 bp, Artificial Sequence
  X2
tttttgcagcagcat

SEQ ID NO: 8 - DNA, 45 bp, Artificial Sequence
  cX2-80-15
aaccaaaaaaagatggtgcaccaatgagaacgggatagtgagaaa

SEQ ID NO: 9 - DNA, 40 bp, Artificial Sequence
  cX2-80-15
tttttttttttttttttttttttttttttttttttttttt

SEQ ID NO: 10 - DNA, 20 bp, Artificial Sequence
  S1T
ttttttttttttttccttcc

SEQ ID NO: 11 - DNA, 576 bp, Artificial Sequence; identical to SEQ ID NO: 2
  the nucleotide sequence encoding the Mnep monomer variant

SEQ ID NO: 12 - DNA, 20 bp, Artificial Sequence
  X
ttcttttcccgtccgctcgt

SEQ ID NO: 13 - DNA, 79 bp, Artificial Sequence
  X
tcgcgcctgtctgcttgtttttttttttctttttttttttctcactatcgcattctcatgcaggtcggtggtcgcagta

SEQ ID NO: 14 - DNA, 20 bp, Artificial Sequence
  S1MC
acgagcggacgggaaaagaa

SEQ ID NO: 15 - DNA, 20 bp, Artificial Sequence
  S1MC
tttttttttttttttttttt

SEQ ID NO: 16 - DNA, 84 bp, Artificial Sequence
  Point mutation primers
ccaccccgaatgtggcactgagtaaatttccgctgtttggcattaccggcattggcggcaaactgccggtgattggcgaaattg

SEQ ID NO: 17 - DNA, 84 bp, Artificial Sequence
  Point mutation primers
caatttcgccaatcaccggcagtttgccgccaatgccggtaatgccaaacagcggaaatttactcagtgccacattcggggtgg